European Patent Specification EP 3 522 718 B1, published July 5, 2023. Title: I DOMAIN CHIMERIC ANTIGEN RECEPTOR SPECIFIC TO ICAM-1. Applicant: Cornell University. The sequence listing filed with the application follows.

SEQUENCE LISTING (1 sequence)

SEQ ID NO: 1 - protein, 1145 aa, Homo sapiens
YNLDVRGARSFSPPRAGRHFGYRVLQVGNGVIVGAPGEGNSTGSLYQCQSGTGHCLPVTLRGSNYTSKYLGMTLATDPTDGSILACDPGLSRTCDQNTYLSGLCYLFRQNLQGPMLQGRPGFQECIKGNVDLVFLFDGSMSLQPDEFQKILDFMKDVMKKLSNTSYQFAAVQFSTSYKTEFDFSDYVKWKDPDALLKHVKHMLLLTNTFGAINYVATEVFREELGARPDATKVLIIITDGEATDSGNIDAAKDIIRYIIGIGKHFQTKESQETLHKFASKPASEFVKILDTFEKLKDLFTELQKKIYVIEGTSKQDLTSFNMELSSSGISADLSRGHAVVGAVGAKDWAGGFLDLKADLQDDTFIGNEPLTPEVRAGYLGYTVTWLPSRQKTSLLASGAPRYQHMGRVLLFQEPQGGGHWSQVQTIHGTQIGSYFGGELCGVDVDQDGETELLLIGAPLFYGEQRGGRVFIYQRRQLGFEEVSELQGDPGYPLGRFGEAITALTDINGDGLVDVAVGAPLEEQGAVYIFNGRHGGLSPQPSQRIEGTQVLSGIQWFGRSIHGVKDLEGDGLADVAVGAESQMIVLSSRPVVDMVTLMSFSPAEIPVHEVECSYSTSNKMKEGVNITICFQIKSLYPQFQGRLVANLTYTLQLDGHRTRRRGLFPGGRHELRRNIAVTTSMSCTDFSFHFPVCVQDLISPINVSLNFSLWEEEGTPRDQRAQGKDIPPILRPSLHSETWEIPFEKNCGEDKKCEANLRVSFSPARSRALRLTAFASLSVELSLSNLEEDAYWVQLDLHFPPGLSFRKVEMLKPHSQIPVSCEELPEESRLLSRALSCNVSSPIFKAGHSVALQMMFNTLVNSSWGDSVELHANVTCNNEDSDLLEDNSATTIIPILYPINILIQDQEDSTLYVSFTPKGPKIHQVKHMYQVRIQPSIHDHNIPTLEAVVGVPQPPSEGPITHQWSVQMEPPVPCHYEDLERLPDAAEPCLPGALFRCPVVFRQEILVQVIGTLELVGEIEASSMFSLCSSLSISFNSSKHFHLYGSNASLAQVVMKVDVVYEKQMLYLYVLSGIGGLLLLLLIFIVLYKVGFFKRNLKEKMEAGRGVPNGIPAEDSEQLASGQEAGDPGCLKPLHEKDSESGGGKD